European Patent Application EP 4 740 958 A1, published May 13, 2026. Title: 一种抗人CCR8的单克隆抗体药物制剂及其用途. Applicant: 齐鲁制药有限公司. Application CN. The sequence listing filed with the application follows.

SEQUENCE LISTING (10 sequences)

SEQ ID NO: 1 - protein, 5 aa, synthetic construct
PFAMN

SEQ ID NO: 2 - protein, 19 aa, synthetic construct
RIRSKANNYATYYADSVKD

SEQ ID NO: 3 - protein, 12 aa, synthetic construct
GRENNYGYAMDY

SEQ ID NO: 4 - protein, 16 aa, synthetic construct
RSSQSLLHSNGITYLY

SEQ ID NO: 5 - protein, 7 aa, synthetic construct
RMSNLAS

SEQ ID NO: 6 - protein, 9 aa, synthetic construct
MQHLTYPFT

SEQ ID NO: 7 - protein, 123 aa, synthetic construct
EVQLVESGGGVVQPGRSLRLSCAASGFPFEPFAMNWVRQAPGKGLEWVARIRSKANNYATYYADSVKDRFAISRDNSKRTLYLLMHSLRFEDTAVYYCVRGRENNYGYAMDYWGQGTTVTVSS

SEQ ID NO: 8 - protein, 112 aa, synthetic construct
DVVMTQSPPSLPVTLGQSASISCRSSQSLLHSNGITYLYWFLQRPGQSPRLLIYRMSNLASGVPDRFSGSGSGTDFTLRISRVEAEDVGVYYCMQHLTYPFTFGIGTKVEIK

SEQ ID NO: 9 - protein, 453 aa, synthetic construct
EVQLVESGGGVVQPGRSLRLSCAASGFPFEPFAMNWVRQAPGKGLEWVARIRSKANNYATYYADSVKDRFAISRDNSKRTLYLLMHSLRFEDTAVYYCVRGRENNYGYAMDYWGQGTTVTVSSASTKGPSVFPLAPSSKSTSGGTAALGCLVKDYFPEPVTVSWNSGALTSGVHTFPAVLQSSGLYSLSSVVTVPSSSLGTQTYICNVNHKPSNTKVDKKVEPKSCDKTHTCPPCPAPELLGGPSVFLFPPKPKDTLMISRTPEVTCVVVDVSHEDPEVKFNWYVDGVEVHNAKTKPREEQYNSTYRVVSVLTVLHQDWLNGKEYKCKVSNKALPAPIEKTISKAKGQPREPQVYTLPPSREEMTKNQVSLTCLVKGFYPSDIAVEWESNGQPENNYKTTPPVLDSDGSFFLYSKLTVDKSRWQQGNVFSCSVMHEALHNHYTQKSLSLSPGK

SEQ ID NO: 10 - protein, 219 aa, synthetic construct
DVVMTQSPPSLPVTLGQSASISCRSSQSLLHSNGITYLYWFLQRPGQSPRLLIYRMSNLASGVPDRFSGSGSGTDFTLRISRVEAEDVGVYYCMQHLTYPFTFGIGTKVEIKRTVAAPSVFIFPPSDEQLKSGTASVVCLLNNFYPREAKVQWKVDNALQSGNSQESVTEQDSKDSTYSLSSTLTLSKADYEKHKVYACEVTHQGLSSPVTKSFNRGEC